European Patent Specification EP 4 352 214 B1, published July 8, 2026. Title: BNovel Type V RNA programmable endonuclease systems. Applicant: Bayer AG. The sequence listing filed with the application follows.

SEQUENCE LISTING (44 sequences)

SEQ ID NO: 1 - protein, 1103 aa, other sequences
  RNA programmable DNA endonuclease B-Gen.1
MTIRSMKLKLKIYSGRSAPQLRQGLWRLHRLLNEGTAYYMDWLVHMRQEALPGKSKEEIRAELERRVRQQQEKNGVQNDQVPMDEVLSALRQLYELLVPSAVNNSGDAQTLSRKFLSPLVDPNSEGGKGTSNAGAKPGWRKKQEAGDPSWEKDYERWLKRKQADPTAEILGKLETAGLKPLFPLYTNEVKDIRWMPLTSKQYVRNWDRDMFQQAIEHLLSWETWNRKVNEERAKLKETVRRFEEQHLANGKDWLSPLQAYEANREQALRDMAISPSDRFRITRRQIKGWSELYERWNKLAPTASVEAYMQEVRHVQKKLGGTFGDADLYRFLAKPENVHIWRDHQERLHYYAAYNDLHKRLMSAKEQAAFTLPDPVAHPLWVRFDARDGNLFTYILQADSSKQRSRRYVNFSRFLWPVEDGYFEETENVKVELALSKQFYRQVIVHDNPTGKQKITFQDYSSKEILEGHLGGAKLQLDRNFLRKSGRDFETGDFGPAFLNVVLDLKPKQEVKNGRLQSPLGQALLVKSRPNDIPKVYGYKPDALAAWLEQASGEESLGSESLRQGFRVMSIDLGVRSAAAISVFSVKGEKTREGDKVCYPVGETGLFAVHDRSFLLRLPGESSEKRVNVERDKRKTERMQIRYHIRTLARVLRLANKATPMDRIKAVQDVLNDIESTRFMNDHDHHVYNHALETLRTYAPDHQGIWEEQVIAAHRQLEHHVGVIVGEWRKNWGKDRRGTVGLSMDNIEELDEMRRLLISWSRRARYPREAKPFQVNESNPVHLLRHLQNLKEDRLKQLANLIVMTALGYVYDSKEKKWKAAYPACQLILFEDLQRYRFHLDRSARENSQLMKWAHRSIPKYVWMQGEPYGLQIGDVWAGFTSRYHAKTGAPGIRCKALTEKDFQQGRLLESLVAEGMFTLQEVGTLKPGDIVPAEGGELFVTLADDSGDRIVITHADINAAQNVQKRFWLANSERFRVACRSVQIASQECFIPSSESVAKKMGKGVFVRDFSFHKDMEVYHWNNQVKLTAKNVPTDHSDDLQDLQDYQAILEEARESSSSYKTLFRDPSGFFFPDDVWVPQNIYWREVKKTITALLRKRIMST

SEQ ID NO: 2 - protein, 1091 aa, other sequences
  RNA programmable DNA endonuclease B-Gen.2
MPIRSFKLKLVTHNGDSTYMDKLRRGLWKTHVIINRGIAYYMNTLALMRQEPYGSKSREEVRLDLLSTLREQQRRNNWSEQTGTDDELLSLSRRVYELLVPSAIGEKGDAQMLSRKFLSPLVDPNSEGGRGTAKSGRKPRWKKMMEEGHPDWEKEKEKDAAKKAEDPTASILADLEAVGLLPLFPLFSDEQKEIRWLPKKKRQFVRTWDRDMFQQALERMLSWESWNRRVAEEYLKLQAQRDEVYAKYLEDAGSWLNDLQTFEKQREEELAEVSFEPNSEYLITRRQIRGWKEVYEKWSKTSENASQEQLWRMVADVQTAMAGAFGDPKVYQFLSQPKHHHIWREHPNRLFYYSKYNEVREKLNRAKKQAAFTLPDPVEHPLWTRFDARGGNIHDYEISKVGKQYHVTFSSLILPEAQSWVEIENVTVGIGNSLQLKRQIRLDGYADKKQKVKYYDYSSRFELTGVLGGAKIQFDRKHLKKAAHRLAEGETGPIFLNVVVDVEPFLEVKNGRLRTPLGQVLQVNTRDWPKVVDYKAKELSVLMENTQIGNENGVSTIEAGMRIMSIDLGQRTAAAVSIFEVISKKPDEKETKLFYPIADTDLYAVHRRSLLLRLPGEEISSKKMIEKRKERARIRSLVRYQIRLLSEVLRLHTQGTAEQRRFKLDELLVSIQKKLELDQSEWISELEKLFDYIDESAEKWKEALVVAHRTLEPIVVEAVRNWKKSLSKENKDRRRIAGISIWSIEELEETRKLLIAWSKHSREPGIPKRLEKEETFAPEHLQHIQNVKDDRLKQMANLFVMTALGYKYDEGNKRWVEAYPACQVILFEDLSRYRFALDRPRRENNRLMKWAHRSIPRLTYMQAELFGIQVGDVYSAYTSRFHAKTGAPGIRCHALTEADLQSNSYVVNQLIKDKFIQDNQTEILKAGQIVPWQGGELFVTFADRSGASLAVIHADINAAQNLQKRFWQHNSEVFRVPCKVVKGGLVPVYEKMRKLFGKGLFVNIDDPESKEVYRWEHSTKMKSKTTPVDLESEDIDHEELSDEWEDMQEGYKTLLRDPSGFFWSSDSWIPQKDFWIRVKSRIGKSLREQIR

SEQ ID NO: 3 - RNA, 106 nt, other sequences
  RNA tracr for B-Gen.1
uaauaaauaauaugaguuacaggcucaugucauuccgugcgugugcugcgaggcucuuacaacgucucaaccacgggaucacguuauuuccacuaagugauuggac

SEQ ID NO: 4 - RNA, 109 nt, other sequences
  RNA tracr for B-Gen.2
cuggauauaauaaagauguuuagcuauaggcuaauaagauaguugugucaagugcuucggagaccuaacacgucauccagucacaacggcuaucuauauuuccacuaac

SEQ ID NO: 5 - DNA, 106 bp, other sequences
  DNA encoding the RNA tracr for B-Gen.1
taataaataatatgagttacaggctcatgtcattccgtgcgtgtgctgcgaggctcttacaacgtctcaaccacgggatcacgttatttccactaagtgattggac

SEQ ID NO: 6 - DNA, 109 bp, other sequences
  DNA encoding the RNA tracr for B-Gen.2
ctggatataataaagatgtttagctataggctaataagatagttgtgtcaagtgcttcggagacctaacacgtcatccagtcacaacggctatctatatttccactaac

SEQ ID NO: 7 - DNA, 8715 bp, other sequences
  Plasmid pBLR373 including the insert for B-GEn.1
gctcagtcctaggtataatgctagctaatacgactcactataggagagaccatggccaccggtctctgctaaagatatgaggagctcaaactggagctgctaacaaagcccgaaaggaagctgagttggctgctgccaccgctgagcaataactagcataaccccttggggcctctaaacgggtcttgaggggttttttgctgaaaggaggaactatatccggattggcgaatgggacgcgccctgtagcggcgcattaagcgcggcgggtgtggtggttacgcgcagcgtgaccgctacacttgccagcgccctagcgcccgctcctttcgctttcttcccttcctttctcgccacgttcgccggctttccccgtcaagctctaaatcgggggctccctttagggttccgatttagtgctttacggcacctcgaccccaaaaaacttgattagggtgatggttcacgtagtgggccatcgccctgatagacggtttttcgccctttgacgttggagtccacgttctttaatagtggactcttgttccaaactggaacaacactcaaccctatctcggtctattcttttgatttataagggattttgccgatttcggcctattggttaaaaaatgagctgatttaacaaaaatttaacgcgaattttaacaaaatattaacgtttacaatttcaggtggcacttttcggggaaatgtgcgcggaacccctatttgtttatttttctaaatacattcaaatatgtatccgctcatgaattaattcttagaaaaactcatcgagcatcaaatgaaactgcaatttattcatatcaggattatcaataccatatttttgaaaaagccgtttctgtaatgaaggagaaaactcaccgaggcagttccataggatggcaagatcctggtatcggtctgcgattccgactcgtccaacatcaatacaacctattaatttcccctcgtcaaaaataaggttatcaagtgagaaatcaccatgagtgacgactgaatccggtgagaatggcaaaagtttatgcatttctttccagacttgttcaacaggccagccattacgctcgtcatcaaaatcactcgcatcaaccaaaccgttattcattcgtgattgcgcctgagcgagacgaaatacgcgatcgctgttaaaaggacaattacaaacaggaatcgaatgcaaccggcgcaggaacactgccagcgcatcaacaatattttcacctgaatcaggatattcttctaatacctggaatgctgttttcccggggatcgcagtggtgagtaaccatgcatcatcaggagtacggataaaatgcttgatggtcggaagaggcataaattccgtcagccagtttagtctgaccatctcatctgtaacatcattggcaacgctacctttgccatgtttcagaaacaactctggcgcatcgggcttcccatacaatcgatagattgtcgcacctgattgcccgacattatcgcgagcccatttatacccatataaatcagcatccatgttggaatttaatcgcggcctagagcaagacgtttcccgttgaatatggctcataacaccccttgtattactgtttatgtaagcagacagttttattgttcatgaccaaaatcccttaacgtgagttttcgttccactgagcgtcagaccccgtagaaaagatcaaaggatcttcttgagatcctttttttctgcgcgtaatctgctgcttgcaaacaaaaaaaccaccgctaccagcggtggtttgtttgccggatcaagagctaccaactctttttccgaaggtaactggcttcagcagagcgcagataccaaatactgtccttctagtgtagccgtagttaggccaccacttcaagaactctgtagcaccgcctacatacctcgctctgctaatcctgttaccagtggctgctgccagtggcgataagtcgtgtcttaccgggttggactcaagacgatagttaccggataaggcgcagcggtcgggctgaacggggggttcgtgcacacagcccagcttggagcgaacgacctacaccgaactgagatacctacagcgtgagctatgagaaagcgccacgcttcccgaagggagaaaggcggacaggtatccggtaagcggcagggtcggaacaggagagcgcacgagggagcttccagggggaaacgcctggtatctttatagtcctgtcgggtttcgccacctctgacttgagcgtcgatttttgtgatgctcgtcaggggggcggagcctatggaaaaacgccagcaacgcggcctttttacggttcctggccttttgctggccttttgctcacatgttctttcctgcgttatcccctgattctgtggataaccgtattaccgcctttgagtgagctgataccgctcgccgcagccgaacgaccgagcgcagcgagtcagtgagcgaggaagcggaagagcgcctgatgcggtattttctccttacgcatctgtgcggtatttcacaccgcatatatggtgcactctcagtacaatctgctctgatgccgcatagttaagccagtatacactccgctatcgctacgtgactgggtcatggctgcgccccgacacccgccaacacccgctgacgcgccctgacgggcttgtctgctcccggcatccgcttacagacaagctgtgaccgtctccgggagctgcatgtgtcagaggttttcaccgtcatcaccgaaacgcgcgaggcagctgcggtaaagctcatcagcgtggtcgtgaagcgattcacagatgtctgcctgttcatccgcgtccagctcgttgagtttctccagaagcgttaatgtctggcttctgataaagcgggccatgttaagggcggttttttcctgtttggtcactgatgcctccgtgtaagggggatttctgttcatgggggtaatgataccgatgaaacgagagaggatgctcacgatacgggttactgatgatgaacatgcccggttactggaacgttgtgagggtaaacaactggcggtatggatgcggcgggaccagagaaaaatcactcagggtcaatgccagcgcttcgttaatacagatgtaggtgttccacagggtagccagcagcatcctgcgatgcagatccggaacataatggtgcagggcgctgacttccgcgtttccagactttacgaaacacggaaaccgaataccattcatgttgttgctcaggtcgcagacgttttgcagcagcagtcgcttcacgttcgctcgcgtatcggtgattcattctgctaaccagtaaggcaaccccgccagcctagccgggtcctcaacgacaggagcacgatcatgcgcacccgtggggccgccatgccggcgataatggcctgcttctcgccgaaacgtttggtggcgggaccagtgacgaaggcttgagcgagggcgtgcaagattccgaataccgcaagcgacaggccgatcatcgtcgcgctccagcgaaagcggtcctcgccgaaaatgacccagagcgctgccggcacctgtcctacgagttgcatgataaagaatacagtcataagtgcggcgacgatagtcatgccccgcgcccaccggaaggagctgactgggttgaaggctctcaagggcatcggtcgagatcccggtgcctaatgagtgagctaacttacattaattgcgttgcgctcactgcccgctttccagtcgggaaacctgtcgtgccagctgcattaatgaatcggccaacgcgcggggagaggcggtttgcgtattgggcgccagggtggtttttcttttcaccagtgagacgggcaacagctgattgcccttcaccgcctggccctgagagagttgcagcaagcggtccacgctggtttgccccagcaggcgaaaatcctgtttgatggtggttaacggcgggatataacatgagctgtattcggtatcgtcgtatcccactaccgagatatccgcaccaacgcgcagcccggactcggtaatggcgcgcattgcgcccagcgccatctgatcgttggcaaccagcatcgcagtgggaacgatgccctcattcagcatttgcatggtttgttgaaaaccggacatggcactccagtcgccttcccgttccgctatcggctgaatttgattgcgagtgagatatttatgccagccagccagacgcagacgcgccgagacagaacttaatgggcccgctaacagcgcgatttgctggtgacccaatgcgaccagatgctccacgcccagtcgcgtaccgtattcatgggagaaaataatactgttgatgggtgtctggtcagagacatcaagaaataacgccggaacattagtgcaggcagcttccacagcaatggcatcctggtcatccagcggatagttaatgatcagcccactgacgcgttgcgcgagaagattgtgcaccgccgctttacaggcttcgacgccgcttcgttctaccatcgacaccaccacgctggcacccagttgatcggcgcgagatttaatcgccgcgacaatttgcgacggcgcgtgcagggccagactggaggtggcaacgccaatcagcaacgactgtttgcccgccagttgttgtgccacgcggttgggaatgtaattcagctccgccatcgccgcttccactttttcccgcgttttcgcagaaacgtggctggcctggttcaccacgcgggaaacggtctgataagagacaccggcatactctgcgacatcgtataacgttactggtttcacattcaccaccctgaattgactctcttccgggcgctatcatgccataccgcgaaaggttttgcgccattcgatggtgtccgggatctcgacgctctcccttatgcgactcctgcattaggaagcagcccagtagtaggttgaggccgttgagcaccgccgccgcaaggaatggtgcatgcaaggagatggcgcccaacagtcccccggccacggggcctgccaccatacccacgccgaaacaagcgctcatgagcccgaagtggcgagcccgatcttccccatcggtgatgtcggcgatataggcgccagcaaccgcacctgtggcgccggtgatgccggccacgatgcgtccggcgtagaggatcgagatctcgatcccgcgaaattaatacgactcactataggggaattgtgagcggataacaattcccctctagatttacactttatgcttccggctcgtatgtttctagagaattcaaataattttgtttaactttaagaaggagatttaaatatgaaaatcgaagaaggtaaaggtcaccaccatcatcaccatatgaccattcgctcgatgaaattaaaactcaagatttactcaggccgctctgcgccgcaattacgccagggtctgtggcgtttacaccgtctgctcaatgaaggcaccgcttattatatggactggttagtacacatgcgtcaagaagccttaccgggcaaatcgaaagaggagattcgtgcggagctggaacgccgtgttcgccagcagcaagagaagaacggcgttcaaaacgatcaagttcccatggatgaggttctgagtgcgctgcgtcagctgtacgaattactggtgcccagtgcggttaacaacagcggcgacgcacagaccctcagccgcaagtttctgagcccgctggtcgacccgaactcggaaggtggcaaaggaaccagcaacgccggtgcaaaaccgggctggcgcaagaagcaagaagcgggcgatcctagctgggaaaaggattacgaacgttggttaaaacgcaagcaggcggatccgacggctgaaattttaggcaaactggaaacggcgggtctgaagccactgttccctctgtacacaaacgaagtgaaagatatccgttggatgccgttaacctcgaaacagtatgtgcgtaactgggatcgcgacatgtttcagcaggcgattgaacatctgttaagctgggaaacctggaaccgcaaggtgaatgaagaacgcgccaaacttaaagaaacagtacgtcgcttcgaagaacagcatttagcgaatggtaaggattggctgagcccactgcaggcatatgaagcaaaccgcgaacaggcgctgcgtgatatggcaatttcgcctagcgaccgttttcgcatcacccgccgtcagattaaaggctggtcggaactttatgaacgttggaacaagctggcgcccacagcgtcagttgaggcatacatgcaagaggtacgtcacgtgcagaagaagctgggcgggacgtttggtgatgcggacttatatcgtttcctggcaaagccggagaatgtgcacatctggcgcgatcatcaggaacgtctgcattattacgcagcgtacaacgaccttcacaaacgccttatgtcggccaaagagcaagcggcctttaccctgccggatccggtggcgcatccgctgtgggtccgcttcgatgcacgtgatggcaaccttttcacctacattctgcaagcggattcatcaaaacagcgctcccgccgctatgttaatttctcccgctttctttggccggtcgaagatggttactttgaagaaaccgaaaacgtgaaagtagaattggcattgtcgaagcagttttatcgccaggttatcgttcatgataaccctacaggcaaacagaaaattacctttcaagattattcgagcaaggaaattctggaaggtcatttgggcggagcgaaactgcaactggatcgcaatttcctgcgtaagtccggacgtgattttgaaacaggtgatttcggaccggcattcttgaacgttgtattagacctcaaaccgaaacaagaggttaagaacggacgcctgcaatctcctctgggccaggcgttactggtgaaaagtcgcccaaacgatatcccgaaagtttacggctataagcctgatgccctggcggcctggttggaacaggcctcgggtgaggaaagtttgggcagtgaaagcctgcgccagggcttccgtgtgatgagtatcgatttaggcgttcgcagtgccgccgcgattagcgttttctctgtgaaaggcgagaaaacccgcgaaggcgataaagtttgttacccggtgggcgaaacgggtctgtttgcggtgcacgaccgtagcttcttattgcgccttccgggagaatcatcagagaaacgtgtgaacgttgagcgtgataaacgtaaaaccgaacgcatgcagattcgctatcatattcgtaccctggcacgcgtactgcgtctggccaataaagcgactcctatggatcgcatcaaagcggtgcaggatgtgctgaacgatattgaaagtacacgttttatgaatgaccacgaccaccatgtgtacaaccatgcactggaaacgctgcgcacttatgcgccggatcatcagggcatctgggaagaacaggtcattgcggcccaccgtcaactggagcatcatgtgggcgtgattgtgggcgaatggcgtaagaactggggcaaagatcgtcgtggaaccgtcggcctgtccatggacaacattgaggaattagacgaaatgcgccgtctgctcatctcatggtcacgtcgcgcgcgttacccgcgcgaagctaaaccatttcaagtcaacgaaagtaacccggtccacctcttacgtcatttgcagaatctcaaagaggatcgcttgaaacaattagctaacttaattgtgatgaccgcgcttggctacgtgtatgacagcaaagagaagaaatggaaagcggcgtatccggcatgccagctgattctgtttgaggatctgcaacgctatcgctttcatctggatcgtagcgcccgtgagaacagccaactgatgaaatgggcgcatcgcagcattccaaaatatgtgtggatgcaaggcgaaccgtatggtctgcagattggagatgtttgggccggttttacctcgcgctaccacgcgaaaaccggtgcccccggcattcgttgcaaagcgttgaccgaaaaggactttcaacagggtcgtctgctggagtcgttggtcgccgaaggtatgttcacgctgcaggaagtaggtactctgaaacctggggatattgtgccggcggaaggtggagaactgtttgtgaccttggcggatgacagtggggatcgtattgtgatcacccatgcggatattaacgcagcgcagaatgtacagaaacgcttttggctcgcgaactcggagcgctttcgcgtggcctgccgctcggtgcagattgccagccaggagtgcttcattcctagcagtgagtcggttgccaagaaaatggggaaaggcgtatttgtgcgcgacttctcgtttcataaggatatggaagtgtatcattggaacaatcaagtcaagctgaccgcaaagaatgtaccgaccgatcattctgacgatctgcaggatctccaggattatcaggcgattcttgaagaggctcgcgaaagttcatcaagctacaaaacgctgtttcgcgatcctagcgggttcttctttccggatgatgtctgggtgccccaaaatatctattggcgtgaagtcaagaaaaccattaccgcgttactgcgtaaacgtattatgagcacttaactcgagtaatgattgacagcta

SEQ ID NO: 8 - DNA, 8679 bp, other sequences
  Plasmid pBLR373 including the insert for B-GEn.2
gctcagtcctaggtataatgctagctaatacgactcactataggagagaccatggccaccggtctctgctaaagatatgaggagctcaaactggagctgctaacaaagcccgaaaggaagctgagttggctgctgccaccgctgagcaataactagcataaccccttggggcctctaaacgggtcttgaggggttttttgctgaaaggaggaactatatccggattggcgaatgggacgcgccctgtagcggcgcattaagcgcggcgggtgtggtggttacgcgcagcgtgaccgctacacttgccagcgccctagcgcccgctcctttcgctttcttcccttcctttctcgccacgttcgccggctttccccgtcaagctctaaatcgggggctccctttagggttccgatttagtgctttacggcacctcgaccccaaaaaacttgattagggtgatggttcacgtagtgggccatcgccctgatagacggtttttcgccctttgacgttggagtccacgttctttaatagtggactcttgttccaaactggaacaacactcaaccctatctcggtctattcttttgatttataagggattttgccgatttcggcctattggttaaaaaatgagctgatttaacaaaaatttaacgcgaattttaacaaaatattaacgtttacaatttcaggtggcacttttcggggaaatgtgcgcggaacccctatttgtttatttttctaaatacattcaaatatgtatccgctcatgaattaattcttagaaaaactcatcgagcatcaaatgaaactgcaatttattcatatcaggattatcaataccatatttttgaaaaagccgtttctgtaatgaaggagaaaactcaccgaggcagttccataggatggcaagatcctggtatcggtctgcgattccgactcgtccaacatcaatacaacctattaatttcccctcgtcaaaaataaggttatcaagtgagaaatcaccatgagtgacgactgaatccggtgagaatggcaaaagtttatgcatttctttccagacttgttcaacaggccagccattacgctcgtcatcaaaatcactcgcatcaaccaaaccgttattcattcgtgattgcgcctgagcgagacgaaatacgcgatcgctgttaaaaggacaattacaaacaggaatcgaatgcaaccggcgcaggaacactgccagcgcatcaacaatattttcacctgaatcaggatattcttctaatacctggaatgctgttttcccggggatcgcagtggtgagtaaccatgcatcatcaggagtacggataaaatgcttgatggtcggaagaggcataaattccgtcagccagtttagtctgaccatctcatctgtaacatcattggcaacgctacctttgccatgtttcagaaacaactctggcgcatcgggcttcccatacaatcgatagattgtcgcacctgattgcccgacattatcgcgagcccatttatacccatataaatcagcatccatgttggaatttaatcgcggcctagagcaagacgtttcccgttgaatatggctcataacaccccttgtattactgtttatgtaagcagacagttttattgttcatgaccaaaatcccttaacgtgagttttcgttccactgagcgtcagaccccgtagaaaagatcaaaggatcttcttgagatcctttttttctgcgcgtaatctgctgcttgcaaacaaaaaaaccaccgctaccagcggtggtttgtttgccggatcaagagctaccaactctttttccgaaggtaactggcttcagcagagcgcagataccaaatactgtccttctagtgtagccgtagttaggccaccacttcaagaactctgtagcaccgcctacatacctcgctctgctaatcctgttaccagtggctgctgccagtggcgataagtcgtgtcttaccgggttggactcaagacgatagttaccggataaggcgcagcggtcgggctgaacggggggttcgtgcacacagcccagcttggagcgaacgacctacaccgaactgagatacctacagcgtgagctatgagaaagcgccacgcttcccgaagggagaaaggcggacaggtatccggtaagcggcagggtcggaacaggagagcgcacgagggagcttccagggggaaacgcctggtatctttatagtcctgtcgggtttcgccacctctgacttgagcgtcgatttttgtgatgctcgtcaggggggcggagcctatggaaaaacgccagcaacgcggcctttttacggttcctggccttttgctggccttttgctcacatgttctttcctgcgttatcccctgattctgtggataaccgtattaccgcctttgagtgagctgataccgctcgccgcagccgaacgaccgagcgcagcgagtcagtgagcgaggaagcggaagagcgcctgatgcggtattttctccttacgcatctgtgcggtatttcacaccgcatatatggtgcactctcagtacaatctgctctgatgccgcatagttaagccagtatacactccgctatcgctacgtgactgggtcatggctgcgccccgacacccgccaacacccgctgacgcgccctgacgggcttgtctgctcccggcatccgcttacagacaagctgtgaccgtctccgggagctgcatgtgtcagaggttttcaccgtcatcaccgaaacgcgcgaggcagctgcggtaaagctcatcagcgtggtcgtgaagcgattcacagatgtctgcctgttcatccgcgtccagctcgttgagtttctccagaagcgttaatgtctggcttctgataaagcgggccatgttaagggcggttttttcctgtttggtcactgatgcctccgtgtaagggggatttctgttcatgggggtaatgataccgatgaaacgagagaggatgctcacgatacgggttactgatgatgaacatgcccggttactggaacgttgtgagggtaaacaactggcggtatggatgcggcgggaccagagaaaaatcactcagggtcaatgccagcgcttcgttaatacagatgtaggtgttccacagggtagccagcagcatcctgcgatgcagatccggaacataatggtgcagggcgctgacttccgcgtttccagactttacgaaacacggaaaccgaataccattcatgttgttgctcaggtcgcagacgttttgcagcagcagtcgcttcacgttcgctcgcgtatcggtgattcattctgctaaccagtaaggcaaccccgccagcctagccgggtcctcaacgacaggagcacgatcatgcgcacccgtggggccgccatgccggcgataatggcctgcttctcgccgaaacgtttggtggcgggaccagtgacgaaggcttgagcgagggcgtgcaagattccgaataccgcaagcgacaggccgatcatcgtcgcgctccagcgaaagcggtcctcgccgaaaatgacccagagcgctgccggcacctgtcctacgagttgcatgataaagaatacagtcataagtgcggcgacgatagtcatgccccgcgcccaccggaaggagctgactgggttgaaggctctcaagggcatcggtcgagatcccggtgcctaatgagtgagctaacttacattaattgcgttgcgctcactgcccgctttccagtcgggaaacctgtcgtgccagctgcattaatgaatcggccaacgcgcggggagaggcggtttgcgtattgggcgccagggtggtttttcttttcaccagtgagacgggcaacagctgattgcccttcaccgcctggccctgagagagttgcagcaagcggtccacgctggtttgccccagcaggcgaaaatcctgtttgatggtggttaacggcgggatataacatgagctgtattcggtatcgtcgtatcccactaccgagatatccgcaccaacgcgcagcccggactcggtaatggcgcgcattgcgcccagcgccatctgatcgttggcaaccagcatcgcagtgggaacgatgccctcattcagcatttgcatggtttgttgaaaaccggacatggcactccagtcgccttcccgttccgctatcggctgaatttgattgcgagtgagatatttatgccagccagccagacgcagacgcgccgagacagaacttaatgggcccgctaacagcgcgatttgctggtgacccaatgcgaccagatgctccacgcccagtcgcgtaccgtattcatgggagaaaataatactgttgatgggtgtctggtcagagacatcaagaaataacgccggaacattagtgcaggcagcttccacagcaatggcatcctggtcatccagcggatagttaatgatcagcccactgacgcgttgcgcgagaagattgtgcaccgccgctttacaggcttcgacgccgcttcgttctaccatcgacaccaccacgctggcacccagttgatcggcgcgagatttaatcgccgcgacaatttgcgacggcgcgtgcagggccagactggaggtggcaacgccaatcagcaacgactgtttgcccgccagttgttgtgccacgcggttgggaatgtaattcagctccgccatcgccgcttccactttttcccgcgttttcgcagaaacgtggctggcctggttcaccacgcgggaaacggtctgataagagacaccggcatactctgcgacatcgtataacgttactggtttcacattcaccaccctgaattgactctcttccgggcgctatcatgccataccgcgaaaggttttgcgccattcgatggtgtccgggatctcgacgctctcccttatgcgactcctgcattaggaagcagcccagtagtaggttgaggccgttgagcaccgccgccgcaaggaatggtgcatgcaaggagatggcgcccaacagtcccccggccacggggcctgccaccatacccacgccgaaacaagcgctcatgagcccgaagtggcgagcccgatcttccccatcggtgatgtcggcgatataggcgccagcaaccgcacctgtggcgccggtgatgccggccacgatgcgtccggcgtagaggatcgagatctcgatcccgcgaaattaatacgactcactataggggaattgtgagcggataacaattcccctctagatttacactttatgcttccggctcgtatgtttctagagaattcaaataattttgtttaactttaagaaggagatttaaatatgaaaatcgaagaaggtaaaggtcaccaccatcatcaccatatgcctattcgctcctttaaactgaaactggtgacacataacggcgatagcacatatatggataaacttcgtcgcggtctgtggaaaacgcacgttatcatcaatcgcggtatcgcctattatatgaacaccctcgcgctgatgcgccaggaaccgtacggctcgaaatctcgtgaagaagtgcgcctggatttgctctcgacgttacgtgaacagcaacgtcgcaataactggtccgagcaaacaggtactgacgatgagctcctttcgctgagtcgccgcgtctacgaactcttggtgccctcggcaatcggcgaaaagggcgacgcgcagatgctgagtcgtaaattcctgagcccgttggttgacccgaatagcgaaggcggccgcggaaccgcgaaaagcggtcgcaaaccgcgttggaagaagatgatggaagaagggcatccggattgggaaaaggagaaagagaaagatgccgcgaagaaggccgaagatccgacagccagtattctcgcggatctcgaagccgtaggccttctgccgctctttcctttgttcagcgacgaacagaaagagatccgctggctccccaagaagaaacgccagtttgtacgtacgtgggatcgcgatatgtttcagcaggccctggaacgtatgctgtcttgggagagttggaaccgccgtgttgcggaagagtacctgaaactgcaggcgcagcgcgatgaggtgtacgcgaagtatctcgaagatgccggctcctggttgaacgatttacagacctttgagaaacagcgtgaagaggagctcgcagaggtgagttttgaaccgaactccgagtacctcatcactcgtcgccagatccgcggttggaaagaagtctatgagaaatggtcgaaaaccagcgaaaatgcctcacaggaacagctgtggcgtatggtggcggacgtgcagaccgcgatggcaggagcatttggagatccaaaagtgtaccagttcttgagccagcctaaacaccaccacatctggcgcgaacacccgaaccgtctgttttactattcgaaatacaatgaagtccgtgagaaattgaaccgcgcaaagaagcaagccgcatttacgctcccggacccggttgaacatccactttggacccgctttgatgcgcgcggcggtaacatccatgactatgaaatcagcaaagtagggaaacagtatcatgttaccttttcgtcactgattcttccggaagcacagagctgggtggaaatcgaaaatgtgacggtcggcattggcaattcactgcaattaaaacgccaaattcgtttagatggttacgctgacaagaaacagaaagtgaagtattacgactatagcagccgcttcgaacttaccggcgtgctgggtggtgcgaagattcagtttgatcgtaaacatctgaagaaggcggcgcaccgcttagctgaaggtgagactggcccgattttcctcaacgtggtagtggacgtggagccctttcttgaagtaaagaacggacgcttgcgtacccctctgggtcaggtgttacaagtgaatacccgtgattggccgaaggttgtcgactacaaagcgaaagaactctcggtgctgatggaaaatacccagatcggtaacgagaatggcgtatccacaattgaagctggaatgcgtattatgagcattgatctgggccagcgcaccgcggctgccgtgtccattttcgaagtaatcagcaagaagccggacgaaaaggaaaccaaattattctatccgatcgctgataccgacctgtacgccgtgcaccgccgcagtttactgctgcgtctgccgggagaggaaattagcagtaagaagatgattgaaaagcgcaaagaacgtgcgcgcatccgtagcttagtgcgctatcagattcgcctgctgagtgaggttctgcgtctgcacacccagggaacggcggagcaacgtcgttttaagctggatgagttgctggtcagcattcagaagaagttagaattggatcaaagtgagtggattagtgaattagaaaagttattcgattatatcgacgaaagcgcggagaagtggaaggaagcactggtagtggcgcaccgcaccttggaaccgattgtggtagaagccgtgcgtaattggaagaagtcactttctaaggaaaataaagaccgccgccgtatcgccggcatttcaatctggagtattgaagaacttgaagaaacgcgtaagttactgattgcttggtccaaacattcccgtgaaccaggaatccctaagcgcctggagaaagaggaaaccttcgcgcctgaacatctgcaacacatccaaaatgttaaggatgatcgtctgaaacagatggcaaacctgtttgttatgacagcgttgggctataaatatgatgaaggcaataagcgctgggttgaggcatacccggcatgccaggtgattctgtttgaggatctcagccgttaccgttttgccctggaccgtccgcgccgcgagaataaccgcttaatgaaatgggcccaccgcagtattccgcgtctgacctacatgcaggccgagctgtttggcattcaagtaggcgatgtttactcagcctacactagccgcttccatgcaaagaccggggcgccgggcatccgctgccacgccctgacagaggcggacctgcaatccaatagctatgtggtaaaccagttgattaaggataaattcatccaagacaatcagaccgaaatcctgaaagcgggccagatcgtcccgtggcagggcggcgaactcttcgtgacgttcgcggatcgcagtggcgccagcttggcagtcattcatgccgacattaatgccgcgcagaatcttcagaaacgcttttggcaacacaactcggaagtgtttcgcgtcccgtgcaaagtggtgaaaggtggcctcgttccggtgtacgagaaaatgcgcaaactgttcgggaaaggattatttgtcaacatcgacgatcccgaaagcaaggaagtgtaccgttgggaacatagcacgaaaatgaaatcaaagacgacccctgtcgatttggagtcagaagatatcgatcacgaggaattaagcgatgagtgggaagatatgcaggaaggctacaagacgctgcttcgcgacccttcgggtttcttttggtcgagtgactcttggattcctcagaaagatttctggattcgcgtgaaaagccgcatcggcaaatcgcttcgcgagcagattcgttaactcgagtaatgattgacagcta

SEQ ID NO: 9 - DNA, 8018 bp, other sequences
  expression construct containing B-Gen.1 with N-terminal linker, a C-terminal linker, T2A-GFP
aaagtagaggaacttcacttcattttgctagaccggtaccgcgttacataacttacggtaaatggcccgcctggctgaccgcccaacgacccccgcccattgacgtcaatagtaacgccaatagggactttccattgacgtcaatgggtggagtatttacggtaaactgcccacttggcagtacatcaagtgtatcatatgccaagtacgccccctattgacgtcaatgacggtaaatggcccgcctggcattgtgcccagtacatgaccttatgggactttcctacttggcagtacatctacgtattagtcatcgctattaccatggtcgaggtgagccccacgttctgcttcactctccccatctcccccccctccccacccccaattttgtatttatttattttttaattattttgtgcagcgatgggggcgggggggggggggcgcgcgccaggtggggcggggcggggcgaggggcggggcggggcgaggcggagaggtgcggcggcagccaatcagagcggcgcgctccgaaagtttccttttatggcgaggcggcggcggcggcggccctataaaaagcgaagcgcgcggcgggcgggagtcgctgcgcgctgccttcgccccgtgccccgctccgccgccgcctcgcgccgcccgccccggctctgactgaccgcgttactcccacaggtgagcgggcgggacggcccttctcctccgggctgtaattagctgagcaagaggtaagggtttaagggatggttggttggtggggtattaatgtttaattacctggagcacctgcctgaaatcactttttttcaggttggcaaccgcggacacccaagcggccgccaatgaagaggcctgccgccacaaagaaggccggccaggccaagaagaagaagggtggcggtggtagtggtggcggtggttcaggcggtggcggctcaggctccatgcctattcgctcttttaagctgaaacttgtaacccataacggcgatagtacgtacatggataaactgcgccgcggcctgtggaaaactcatgtgataataaaccgcggcatcgcgtactacatgaacaccttggccctcatgaggcaagaaccctacgggtccaagagccgggaagaagtacggttggatctgctttccactctgagagagcagcaacgccggaacaattggtcagaacaaaccgggactgatgatgaattgctttccctgagccgtcgagtttacgagcttcttgtaccatccgctataggtgaaaagggcgatgcgcaaatgctgagccgcaaatttctctcccctctcgtggacccaaacagtgagggcgggcgcgggaccgccaaaagtgggagaaagccacggtggaagaagatgatggaagaaggacaccccgactgggaaaaggagaaggaaaaggatgcggctaagaaggcagaggatccaacagcatctatattggcggatctcgaggcagtgggactgttgccacttttcccgctgttttctgacgaacagaaagaaatccgctggctccccaagaagaagcgtcagtttgtgaggacatgggaccgggatatgttccaacaggcccttgaacgaatgctgagctgggaaagctggaatcgcagagttgccgaggaatacttgaagctccaggcccagcgggacgaggtgtatgccaaataccttgaggatgctggctcctggcttaatgatctgcagactttcgaaaagcagcgcgaagaggaactggcggaagtaagcttcgaacccaactctgagtacctgattactcgccggcagattcgcgggtggaaggaagtgtatgaaaagtggtcaaagaccagcgaaaatgcgagccaggagcagttgtggcggatggtggctgacgtgcagactgccatggccggcgcgttcggagatcccaaagtgtaccagtttctttctcagcctaagcaccaccatatttggagagagcatccaaatagactgttctactacagcaagtacaacgaggtccgggagaagctcaacagggccaagaagcaggcggcctttaccctgccagatcccgtggagcacccactgtggacacgttttgatgcgcgcggcggcaatatccatgactacgagatatccaaggtgggcaagcaataccacgtgacgttcagctctcttatcctgccagaggcccagagttgggtggagattgagaatgttacagtgggtatcgggaacagcctgcagctgaaacgccagattcgcttggacggttacgcagacaagaagcagaaagtcaaatattatgattattccagcaggttcgagctcacaggagtactcggcggagcaaagatccaattcgataggaagcatcttaagaaggctgctcacagactggctgagggcgaaacagggccgatcttcttgaatgttgtggtggatgtagaaccattcttggaagtgaagaatggacgtttgcggactccactcggtcaagtcctgcaggtgaacactagagattggcccaaggtcgtcgactacaaagcaaaggagctgtcagtcttgatggaaaacacgcaaattggcaacgagaatggggtgtctacaatcgaggccggaatgaggattatgtctattgacctgggacagaggaccgctgctgccgtgtctattttcgaggtcatttctaagaaacctgacgaaaaggaaacgaagctgttttatcccatcgcagacacagatctgtatgccgttcacaggcgaagtctcctgctgagattgcccggcgaggagatctctagtaagaaaatgattgagaagcggaaagagcgcgcacgtatccgctccctggtgaggtatcagatcaggctcctctcagaagtcctgcggcttcacacacagggcaccgctgaacagcgtcggtttaagctggacgagctgctcgtgagcatccagaagaagttggagcttgaccagagcgagtggatttcagaactcgagaaactcttcgactatatcgatgagtcagctgagaaatggaaagaggctctggtcgtggctcacagaactctggagcctatcgtggttgaagccgtcagaaactggaagaagtctctgtccaaagaaaacaaggatagacgcaggattgccggaatctccatctggtctatagaggagctcgaggaaacccgcaagctgcttattgcatggtctaaacactccagagaacctggcattccgaaaagacttgagaaagaggaaacatttgctccagaacacctgcagcacatacagaacgtgaaagacgatcgccttaaacagatggctaacttgtttgtgatgaccgccttgggctataagtatgatgaaggcaataagcggtgggtggaagcgtatccagcatgccaggtaatcctgtttgaggatttgtctagatatcggttcgccctggacagacctaggcgggagaacaatcgattgatgaagtgggcccaccgcagtatcccaaggctcacctacatgcaggctgaactgtttggaatccaggtgggcgatgtctattcagcgtacacctctagattccacgccaaaacaggggcccccgggatccgctgtcatgcactgacagaagccgatcttcaatctaatagttacgttgtgaaccagctgataaaggataaatttattcaagacaaccagactgaaatcctcaaggccggccagatagttccttggcagggcggtgagttgtttgttacctttgcagatagatccggcgccagcttggctgttatccacgccgatattaatgcagcgcagaaccttcagaaaaggttttggcagcacaactcagaggtgttccgagtgccttgtaaggtggtgaagggcgggttggtccctgtttatgaaaagatgcgaaagcttttcggaaaaggcctctttgtaaatatagacgacccagaatccaaggaagtctaccgctgggaacattccactaagatgaaatccaagactacaccagttgaccttgaaagcgaagatattgatcacgaggaactcagcgacgagtgggaagatatgcaggaaggatacaaaacactgctgcgtgacccttcaggcttcttctggtcctcagacagttggatccctcagaaggatttctggatcagagtcaagagcagaatcggcaagtctctgcgggagcagattcgcggtggaagcggaggcagcgggggatcaggtccccctaagaaaaagcggaaggtgggcggtggcggcggttcacatcatcatcaccatcatggcggtgaaggacgcggctcccttctgacctgtggtgacgtggaagagaaccccggccctgaattcatgtctggcggcgaggaactgtttgccggaatcgtgcctgtgctgatcgagctggatggggatgtgcacggccacaagtttagcgtcagaggcgaaggcgaaggggacgccgattacggcaagctggaaatcaagttcatctgcaccaccggaaagctgcccgtgccttggcctacactggtcaccacactgtgctacggcatccagtgcttcgccagatatcccgagcatatgaagatgaacgacttcttcaagagcgccatgcctgagggctacatccaagagcggacaatccagttccaggacgacggcaagtacaagaccaggggcgaagtgaagttcgagggcgacaccctggtcaacagaatcgagctgaagggcaaagacttcaaagaggacggcaacatcctgggccacaagcttgagtacagcttcaacagccacaacgtgtacatcagacccgacaaggccaacaacggcctggaagccaacttcaagacccggcacaacatcgaaggtggcggagtgcagctggccgatcactaccagacaaatgtgcccctcggagatggccccgtgctgatccctatcaaccactacctgagcacccagaccaagatcagcaaggacagaaacgaggcccgggaccacatggtgctgctggaaagctttagcgcctgctgtcacacccacggcatggacgagctgtacagataatgactcgagatcagcctcgactgtgccttctagttgccagccatctgttgtttgcccctcccccgtgccttccttgaccctggaaggtgccactcccactgtcctttcctaataaaatgaggaaattgcatccccacttcagaagttcctatactttctaatgagtgagctaactcacattaattgcgttgcgctcactgcccgctttccagtcgggaaacctgtcgtgccagctgcattaatgaatcggccaacgcgcggggagaggcggtttgcgtattgggcgctcttgcgcttcctcgctcactgactcgctgcgctcggtcgttcggctgcggcgagcggtatcagctcactcaaaggcggtaatacggttatccacagaatcaggggataacgcaggaaagaacatgtgagcaaaaggccagcaaaaggccaggaaccgtaaaaaggccgcgttgctggcgtttttccataggctccgcccccctgacgagcatcacaaaaatcgacgctcaagtcagaggtggcgaaacccgacaggactataaagataccaggcgtttccccctggaagctccctcgtgcgctctcctgttccgaccctgccgcttaccggatacctgtccgcctttctcccttcgggaagcgtggcgctttctcatagctcacgctgtaggtatctcagttcggtgtaggtcgttcgctccaagctgggctgtgtgcacgaaccccccgttcagcccgaccgctgcgccttatccggtaactatcgtcttgagtccaacccggtaagacacgacttatcgccactggcagcagccactggtaacaggattagcagagcgaggtatgtaggcggtgctacagagttcttgaagtggtggcctaactacggctacactagaagaacagtatttggtatctgcgctctgctgaagccagttaccttcggaaaaagagttggtagctcttgatccggcaaacaaaccaccgctggtagcggtggtttttttgtttgcaagcagcagattacgcgcagaaaaaaaggatctcaagaagatcctttgatcttttctacggggtctgacgctcagtggaacgaaaactcacgttaagggattttggtcatgagattatcaaaaaggatcttcacctagatccttttaaattaaaaatgaagttttaaatcaatctaaagtatatatgagtaaacttggtctgacagttaccaatgcttaatcagtgaggcacctatctcagcgatctgtctatttcgttcatccatagttgcctgactccccgtcgtgtagataactacgatacgggagggcttaccatctggccccagtgctgcaatgataccgcgtgacccacgctcaccggctccagatttatcagcaataaaccagccagccggaagggccgagcgcagaagtggtcctgcaactttatccgcctccatccagtctattaattgttgccgggaagctagagtaagtagttcgccagttaatagtttgcgcaacgttgttgccattgctacaggcatcgtggtgtcacgctcgtcgtttggtatggcttcattcagctccggttcccaacgatcaaggcgagttacatgatcccccatgttgtgcaaaaaagcggttagctccttcggtcctccgatcgttgtcagaagtaagttggccgcagtgttatcactcatggttatggcagcactgcataattctcttactgtcatgccatccgtaagatgcttttctgtgactggtgagtactcaaccaagtcattctgagaatagtgtatgcggcgaccgagttgctcttgcccggcgtcaatacgggataataccgcgccacatagcagaactttaaaagtgctcatcattggaaaacgttcttcggggcgaaaactctcaaggatcttaccgctgttgagatccagttcgatgtaacccactcgtgcacccaactgatcttcagcatcttttactttcaccagcgtttctgggtgagcaaaaacaggaaggcaaaatgccgcaaaaaagggaataagggcgacacggaaatgttgaatactcatactcttcctttttcaatattattgaagcatttatcagggttattgtctcatgagcggatacatatttgaatgtatttagaaaaataaacaaataggggttccgcgcatatttccccgaaaagtgccacctgacgtcgacggatcgggagatctcccgatcccctatggtgcactctcagtacaatctgctctgatgccgcatagttaagccagtatctgctccctgcttgtgtgttggaggtcgctgagtagtgcgcgagcaaaatttaagctacaacaaggcaaggcttgaccgaacaaactctttctgtgttgtaaaacgacggccagtcttaagctcgggccccctgggcggttctgataacgagtaatcgttaatccgcaaataacgtaaaaacccgcttcggcgggtttttttatggggggagtttagggaaagagcatttgtcagaatatttaagggcgcctgtcactttgcttgatatatgagaattatttaaccttataaatgagaaaaaagcaacgcactttaaataagatacgttgctttttcgattgatgaacacctataattaaactattcatctattatttatgattttttgtatatacaatatttctagtttgttaaagagaattaagaaaataaatctcgaaaataataaagggaaaatcagtttttgatatcaaaattatacatgtcaacgataatacaaaatataatacaaactataagatgttatcagtatttattatgcatttagaataaattttgtgtcgcccttattcgactcactatagaagttcctattctctag

SEQ ID NO: 10 - DNA, 8054 bp, other sequences
  expression construct containing B-Gen.2 with N-terminal linker, a C-terminal linker, T2A-GFP
ctctagaaagtagaggaacttcacttcattttgctagaccggtaccgcgttacataacttacggtaaatggcccgcctggctgaccgcccaacgacccccgcccattgacgtcaatagtaacgccaatagggactttccattgacgtcaatgggtggagtatttacggtaaactgcccacttggcagtacatcaagtgtatcatatgccaagtacgccccctattgacgtcaatgacggtaaatggcccgcctggcattgtgcccagtacatgaccttatgggactttcctacttggcagtacatctacgtattagtcatcgctattaccatggtcgaggtgagccccacgttctgcttcactctccccatctcccccccctccccacccccaattttgtatttatttattttttaattattttgtgcagcgatgggggcgggggggggggggcgcgcgccaggtggggcggggcggggcgaggggcggggcggggcgaggcggagaggtgcggcggcagccaatcagagcggcgcgctccgaaagtttccttttatggcgaggcggcggcggcggcggccctataaaaagcgaagcgcgcggcgggcgggagtcgctgcgcgctgccttcgccccgtgccccgctccgccgccgcctcgcgccgcccgccccggctctgactgaccgcgttactcccacaggtgagcgggcgggacggcccttctcctccgggctgtaattagctgagcaagaggtaagggtttaagggatggttggttggtggggtattaatgtttaattacctggagcacctgcctgaaatcactttttttcaggttggcaaccgcggacacccaagcggccgccaatgaagaggcctgccgccacaaagaaggccggccaggccaagaagaagaagggtggcggtggtagtggtggcggtggttcaggcggtggcggctcaggctccatgaccatcagaagtatgaagctgaagcttaaaatctatagcggcaggtccgcgccccaactcaggcagggtctgtggcgtttgcatcggctgttgaacgagggaacggcctattacatggattggcttgtacatatgagacaagaggctctcccaggcaaaagcaaagaagagattagagctgaattggagagaagagtgagacagcagcaggaaaagaatggtgtgcaaaatgaccaggtcccgatggacgaagtcctcagcgcacttaggcaactgtatgagcttctggtcccgtctgccgtaaataattccggcgacgcacagacgctgtctaggaagttcttgtctccattggtggacccaaactccgagggtggaaagggcacgtcaaacgccggagccaagcctggctggcggaagaaacaagaggcaggggacccaagctgggagaaagactatgagagatggctcaaacgcaagcaggctgaccctaccgctgagattttgggtaagctggaaaccgccggcctcaaacccctcttccccctgtacacaaatgaagtcaaggatataaggtggatgccactgacgtctaaacaatatgtccgaaactgggatcgcgatatgttccaacaagctatcgagcatctgctcagttgggaaacttggaatagaaaggtgaatgaggaaagggcgaaactgaaggaaacagtcaggcgctttgaagaacagcacctggccaatggaaaggattggctctccccacttcaggcctatgaagccaatcgagaacaggcacttagagacatggccatatctcctagcgatcgcttcaggatcactaggcgccaaataaagggatggtctgagctttatgaaaggtggaacaagctcgcacctaccgctagcgtagaggcgtacatgcaggaagttcgccatgtacagaagaaactcggcggtacctttggagatgccgacctctaccggtttctggccaaacccgagaacgtgcacatatggcgcgaccaccaggagcggctgcactactatgccgcatacaatgatttgcataagcgactcatgagcgccaaagagcaggctgcttttacactccccgaccctgtggcccatccactgtgggtgcgctttgacgccagagatggcaatctgtttacttacatactgcaggccgactcttcaaagcagaggtcacgtagatacgtcaatttctctcgttttctgtggcctgttgaagatgggtactttgaggaaacggagaacgtcaaagttgagctggctctgtccaagcaattttatagacaggtgattgtccacgacaacccaacgggaaagcagaagataacgttccaggattactccagtaaagaaatcctcgaagggcatcttggcggggccaaactgcagctcgaccggaatttccttcggaaatcagggcgggactttgagacaggcgattttgggccggcttttctgaacgtggtgttggacctgaagccaaaacaggaagtgaagaatgggcgcttgcagtcccctcttggccaggcgttgctcgttaaaagcagacccaacgatatcccgaaggtgtacggatacaaaccagatgcattggcagcttggctggagcaagccagtggtgaagagtccctggggagcgagtcattgcgtcaggggtttagagtaatgtcaattgatctcggcgtcaggtctgccgctgctatatccgtctttagtgtgaaaggagagaaaacccgtgagggcgataaggtgtgctatccagttggggagacaggcctcttcgccgtccacgataggtcttttctgctcagactcccgggtgaatcaagcgagaagcgggtgaatgtggagcgtgataaacgtaagacagagagaatgcagatccgttatcacatcaggaccctggcgcgcgtgttgagactcgcaaacaaggcaaccccaatggaccggatcaaggccgtgcaggatgtgctgaacgatatcgagtctactaggttcatgaatgaccatgaccaccacgtttacaaccatgctctcgaaaccctcagaacctacgctcctgatcaccaggggatctgggaagaacaagtaatcgccgcccatcgccagctcgaacaccacgtcggcgttatcgtaggggagtggcggaagaactggggtaaagatcgtcgagggacagtcgggctgagcatggacaacattgaagaactcgatgagatgaggagattgctgatctcttggagccgccgggctcgttaccctcgcgaggcgaagcctttccaagtgaacgagtcaaaccctgtgcacctgttgcggcatctgcagaatttgaaagaggacagactgaagcagcttgccaacctgattgtgatgaccgccctgggctatgtgtacgactccaaggaaaagaagtggaaagctgcataccctgcatgccagctgatccttttcgaggacctgcagaggtacaggttccacctcgaccgtagtgccagggaaaactcacagctgatgaaatgggcacataggtcaatcccaaagtatgtgtggatgcagggtgagccctacggacttcaaatcggcgatgtgtgggcaggcttcacttcccggtaccacgcgaaaaccggggctcccggaattcggtgtaaagcactgaccgaaaaggattttcagcagggccgacttctggagtcactcgtcgcggaaggcatgtttaccctgcaggaagtgggcacgttgaaaccaggggacatcgttcccgcggaaggcggcgaacttttcgtgactctggccgatgactctggagacaggatcgtcatcacccacgcagatattaacgcagctcagaatgtccagaagcgattttggctcgcaaatagcgagaggttccgcgttgcatgtcgcagcgtgcaaatcgcatcccaggagtgttttattccttccagcgagtctgtcgccaagaagatgggcaagggagtctttgtgcgggacttctcctttcacaaagacatggaagtgtaccactggaataaccaggtcaagctcacagcaaagaacgtaccgaccgaccacagcgatgatctccaggacctgcaggactaccaggctatcctcgaagaagccagggagtctagtagcagctacaagacgctgtttagggatccttctgggttcttcttcccagacgatgtgtgggtccctcagaatatttactggcgagaggttaagaaaacaatcaccgctctgctgcgtaagcgcatcatgtccaccggtggaagcggaggcagcgggggatcaggtccccctaagaaaaagcggaaggtgggcggtggcggcggttcacatcatcatcaccatcatggcggtgaaggacgcggctcccttctgacctgtggtgacgtggaagagaaccccggccctgaattcatgtctggcggcgaggaactgtttgccggaatcgtgcctgtgctgatcgagctggatggggatgtgcacggccacaagtttagcgtcagaggcgaaggcgaaggggacgccgattacggcaagctggaaatcaagttcatctgcaccaccggaaagctgcccgtgccttggcctacactggtcaccacactgtgctacggcatccagtgcttcgccagatatcccgagcatatgaagatgaacgacttcttcaagagcgccatgcctgagggctacatccaagagcggacaatccagttccaggacgacggcaagtacaagaccaggggcgaagtgaagttcgagggcgacaccctggtcaacagaatcgagctgaagggcaaagacttcaaagaggacggcaacatcctgggccacaagcttgagtacagcttcaacagccacaacgtgtacatcagacccgacaaggccaacaacggcctggaagccaacttcaagacccggcacaacatcgaaggtggcggagtgcagctggccgatcactaccagacaaatgtgcccctcggagatggccccgtgctgatccctatcaaccactacctgagcacccagaccaagatcagcaaggacagaaacgaggcccgggaccacatggtgctgctggaaagctttagcgcctgctgtcacacccacggcatggacgagctgtacagataatgactcgagatcagcctcgactgtgccttctagttgccagccatctgttgtttgcccctcccccgtgccttccttgaccctggaaggtgccactcccactgtcctttcctaataaaatgaggaaattgcatccccacttcagaagttcctatactttctaatgagtgagctaactcacattaattgcgttgcgctcactgcccgctttccagtcgggaaacctgtcgtgccagctgcattaatgaatcggccaacgcgcggggagaggcggtttgcgtattgggcgctcttgcgcttcctcgctcactgactcgctgcgctcggtcgttcggctgcggcgagcggtatcagctcactcaaaggcggtaatacggttatccacagaatcaggggataacgcaggaaagaacatgtgagcaaaaggccagcaaaaggccaggaaccgtaaaaaggccgcgttgctggcgtttttccataggctccgcccccctgacgagcatcacaaaaatcgacgctcaagtcagaggtggcgaaacccgacaggactataaagataccaggcgtttccccctggaagctccctcgtgcgctctcctgttccgaccctgccgcttaccggatacctgtccgcctttctcccttcgggaagcgtggcgctttctcatagctcacgctgtaggtatctcagttcggtgtaggtcgttcgctccaagctgggctgtgtgcacgaaccccccgttcagcccgaccgctgcgccttatccggtaactatcgtcttgagtccaacccggtaagacacgacttatcgccactggcagcagccactggtaacaggattagcagagcgaggtatgtaggcggtgctacagagttcttgaagtggtggcctaactacggctacactagaagaacagtatttggtatctgcgctctgctgaagccagttaccttcggaaaaagagttggtagctcttgatccggcaaacaaaccaccgctggtagcggtggtttttttgtttgcaagcagcagattacgcgcagaaaaaaaggatctcaagaagatcctttgatcttttctacggggtctgacgctcagtggaacgaaaactcacgttaagggattttggtcatgagattatcaaaaaggatcttcacctagatccttttaaattaaaaatgaagttttaaatcaatctaaagtatatatgagtaaacttggtctgacagttaccaatgcttaatcagtgaggcacctatctcagcgatctgtctatttcgttcatccatagttgcctgactccccgtcgtgtagataactacgatacgggagggcttaccatctggccccagtgctgcaatgataccgcgtgacccacgctcaccggctccagatttatcagcaataaaccagccagccggaagggccgagcgcagaagtggtcctgcaactttatccgcctccatccagtctattaattgttgccgggaagctagagtaagtagttcgccagttaatagtttgcgcaacgttgttgccattgctacaggcatcgtggtgtcacgctcgtcgtttggtatggcttcattcagctccggttcccaacgatcaaggcgagttacatgatcccccatgttgtgcaaaaaagcggttagctccttcggtcctccgatcgttgtcagaagtaagttggccgcagtgttatcactcatggttatggcagcactgcataattctcttactgtcatgccatccgtaagatgcttttctgtgactggtgagtactcaaccaagtcattctgagaatagtgtatgcggcgaccgagttgctcttgcccggcgtcaatacgggataataccgcgccacatagcagaactttaaaagtgctcatcattggaaaacgttcttcggggcgaaaactctcaaggatcttaccgctgttgagatccagttcgatgtaacccactcgtgcacccaactgatcttcagcatcttttactttcaccagcgtttctgggtgagcaaaaacaggaaggcaaaatgccgcaaaaaagggaataagggcgacacggaaatgttgaatactcatactcttcctttttcaatattattgaagcatttatcagggttattgtctcatgagcggatacatatttgaatgtatttagaaaaataaacaaataggggttccgcgcatatttccccgaaaagtgccacctgacgtcgacggatcgggagatctcccgatcccctatggtgcactctcagtacaatctgctctgatgccgcatagttaagccagtatctgctccctgcttgtgtgttggaggtcgctgagtagtgcgcgagcaaaatttaagctacaacaaggcaaggcttgaccgaacaaactctttctgtgttgtaaaacgacggccagtcttaagctcgggccccctgggcggttctgataacgagtaatcgttaatccgcaaataacgtaaaaacccgcttcggcgggtttttttatggggggagtttagggaaagagcatttgtcagaatatttaagggcgcctgtcactttgcttgatatatgagaattatttaaccttataaatgagaaaaaagcaacgcactttaaataagatacgttgctttttcgattgatgaacacctataattaaactattcatctattatttatgattttttgtatatacaatatttctagtttgttaaagagaattaagaaaataaatctcgaaaataataaagggaaaatcagtttttgatatcaaaattatacatgtcaacgataatacaaaatataatacaaactataagatgttatcagtatttattatgcatttagaataaattttgtgtcgcccttattcgactcactatagaagttcctatt

SEQ ID NO: 11 - DNA, 164 bp, other sequences
  ATTA PAM containing guide sequence
gctggatataataaagatgtttagctataggctaataagatagttgtgtcaagtgcttcggagacctaacacgtcatccagtcacaacggctatctatatttccactaacaaaagttagtggaaatgtagatggttagcactggacaagtagcaagaaattaat

SEQ ID NO: 12 - DNA, 164 bp, other sequences
  ATTT PAM containing guide sequence
gctggatataataaagatgtttagctataggctaataagatagttgtgtcaagtgcttcggagacctaacacgtcatccagtcacaacggctatctatatttccactaacaaaagttagtggaaatgtagatggttagcacgttttctttagttattaatttct

SEQ ID NO: 13 - DNA, 164 bp, other sequences
  ATTC PAM containing guide sequence
gctggatataataaagatgtttagctataggctaataagatagttgtgtcaagtgcttcggagacctaacacgtcatccagtcacaacggctatctatatttccactaacaaaagttagtggaaatgtagatggttagcaccattaactagcattataatgcac

SEQ ID NO: 14 - DNA, 164 bp, other sequences
  ATTG PAM containing guide sequence
gctggatataataaagatgtttagctataggctaataagatagttgtgtcaagtgcttcggagacctaacacgtcatccagtcacaacggctatctatatttccactaacaaaagttagtggaaatgtagatggttagcactttagtgactgtaattttctttt

SEQ ID NO: 15 - DNA, 164 bp, other sequences
  ATTT PAM containing guide sequence
gctggatataataaagatgtttagctataggctaataagatagttgtgtcaagtgcttcggagacctaacacgtcatccagtcacaacggctatctatatttccactaacaaaagttagtggaaatgtagatggttagcacgtgaagtcttacaaggttatctt

SEQ ID NO: 16 - DNA, 164 bp, other sequences; identical to SEQ ID NO: 14
  ATTG PAM containing guide sequence

SEQ ID NO: 17 - DNA, 164 bp, other sequences
  ATTC PAM containing guide sequence
gctggatataataaagatgtttagctataggctaataagatagttgtgtcaagtgcttcggagacctaacacgtcatccagtcacaacggctatctatatttccactaacaaaagttagtggaaatgtagatggttagcacaatcttcaaccctattctgtgaa

SEQ ID NO: 18 - DNA, 164 bp, other sequences
  ATTA PAM containing guide sequence
gctggatataataaagatgtttagctataggctaataagatagttgtgtcaagtgcttcggagacctaacacgtcatccagtcacaacggctatctatatttccactaacaaaagttagtggaaatgtagatggttagcacataactaaagaaaacaaatctta

SEQ ID NO: 19 - DNA, 164 bp, other sequences
  GTTA PAM containing guide sequence
gctggatataataaagatgtttagctataggctaataagatagttgtgtcaagtgcttcggagacctaacacgtcatccagtcacaacggctatctatatttccactaacaaaagttagtggaaatgtagatggttagcacgtacagttttgctgaaaggttat

SEQ ID NO: 20 - DNA, 164 bp, other sequences
  GTTC PAM containing guide sequence
gctggatataataaagatgtttagctataggctaataagatagttgtgtcaagtgcttcggagacctaacacgtcatccagtcacaacggctatctatatttccactaacaaaagttagtggaaatgtagatggttagcactgcttattatggacaagtagcaa

SEQ ID NO: 21 - DNA, 164 bp, other sequences
  GTTT PAM containing guide sequence
gctggatataataaagatgtttagctataggctaataagatagttgtgtcaagtgcttcggagacctaacacgtcatccagtcacaacggctatctatatttccactaacaaaagttagtggaaatgtagatggttagcactattccattaactagcattataa

SEQ ID NO: 22 - DNA, 164 bp, other sequences
  GTTT PAM containing guide sequence
gctggatataataaagatgtttagctataggctaataagatagttgtgtcaagtgcttcggagacctaacacgtcatccagtcacaacggctatctatatttccactaacaaaagttagtggaaatgtagatggttagcaccagtgcgacgccgcgagccccga

SEQ ID NO: 23 - DNA, 164 bp, other sequences
  GTTG PAM containing guide sequence
gctggatataataaagatgtttagctataggctaataagatagttgtgtcaagtgcttcggagacctaacacgtcatccagtcacaacggctatctatatttccactaacaaaagttagtggaaatgtagatggttagcacgacgaaaagtttcagtgcgacgc

SEQ ID NO: 24 - DNA, 164 bp, other sequences
  GTTC PAM containing guide sequence
gctggatataataaagatgtttagctataggctaataagatagttgtgtcaagtgcttcggagacctaacacgtcatccagtcacaacggctatctatatttccactaacaaaagttagtggaaatgtagatggttagcactcgcttcggaggagccgtggtcc

SEQ ID NO: 25 - DNA, 170 bp, other sequences
  ATTA PAM containing guide sequence
gtaataaataatatgagttacaggctcatgtcattccgtgcgtgtgctgcgaggctcttacaacgtctcaaccacgggatcacgttatttccactaagtgattggacaaaagtcagattatttagtggaaagtaacgtgattagcactggacaagtagcaagaaattaat

SEQ ID NO: 26 - DNA, 170 bp, other sequences
  ATTT PAM containing guide sequence
gtaataaataatatgagttacaggctcatgtcattccgtgcgtgtgctgcgaggctcttacaacgtctcaaccacgggatcacgttatttccactaagtgattggacaaaagtcagattatttagtggaaagtaacgtgattagcacgttttctttagttattaatttct

SEQ ID NO: 27 - DNA, 170 bp, other sequences
  ATTC PAM containing guide sequence
gtaataaataatatgagttacaggctcatgtcattccgtgcgtgtgctgcgaggctcttacaacgtctcaaccacgggatcacgttatttccactaagtgattggacaaaagtcagattatttagtggaaagtaacgtgattagcaccattaactagcattataatgcac

SEQ ID NO: 28 - DNA, 170 bp, other sequences
  ATTG PAM containing guide sequence
gtaataaataatatgagttacaggctcatgtcattccgtgcgtgtgctgcgaggctcttacaacgtctcaaccacgggatcacgttatttccactaagtgattggacaaaagtcagattatttagtggaaagtaacgtgattagcactttagtgactgtaattttctttt

SEQ ID NO: 29 - DNA, 170 bp, other sequences
  ATTT PAM containing guide sequence
gtaataaataatatgagttacaggctcatgtcattccgtgcgtgtgctgcgaggctcttacaacgtctcaaccacgggatcacgttatttccactaagtgattggacaaaagtcagattatttagtggaaagtaacgtgattagcacgtgaagtcttacaaggttatctt

SEQ ID NO: 30 - DNA, 170 bp, other sequences; identical to SEQ ID NO: 28
  ATTG PAM containing guide sequence

SEQ ID NO: 31 - DNA, 170 bp, other sequences
  ATTC PAM containing guide sequence
gtaataaataatatgagttacaggctcatgtcattccgtgcgtgtgctgcgaggctcttacaacgtctcaaccacgggatcacgttatttccactaagtgattggacaaaagtcagattatttagtggaaagtaacgtgattagcacaatcttcaaccctattctgtgaa

SEQ ID NO: 32 - DNA, 170 bp, other sequences
  ATTA PAM containing guide sequence
gtaataaataatatgagttacaggctcatgtcattccgtgcgtgtgctgcgaggctcttacaacgtctcaaccacgggatcacgttatttccactaagtgattggacaaaagtcagattatttagtggaaagtaacgtgattagcacataactaaagaaaacaaatctta

SEQ ID NO: 33 - DNA, 170 bp, other sequences
  GTTA PAM containing guide sequence
gtaataaataatatgagttacaggctcatgtcattccgtgcgtgtgctgcgaggctcttacaacgtctcaaccacgggatcacgttatttccactaagtgattggacaaaagtcagattatttagtggaaagtaacgtgattagcacgtacagttttgctgaaaggttat

SEQ ID NO: 34 - DNA, 170 bp, other sequences
  GTTC PAM containing guide sequence
gtaataaataatatgagttacaggctcatgtcattccgtgcgtgtgctgcgaggctcttacaacgtctcaaccacgggatcacgttatttccactaagtgattggacaaaagtcagattatttagtggaaagtaacgtgattagcactgcttattatggacaagtagcaa

SEQ ID NO: 35 - DNA, 170 bp, other sequences
  GTTT PAM containing guide sequence
gtaataaataatatgagttacaggctcatgtcattccgtgcgtgtgctgcgaggctcttacaacgtctcaaccacgggatcacgttatttccactaagtgattggacaaaagtcagattatttagtggaaagtaacgtgattagcactattccattaactagcattataa

SEQ ID NO: 36 - DNA, 170 bp, other sequences
  GTTT PAM containing guide sequence
gtaataaataatatgagttacaggctcatgtcattccgtgcgtgtgctgcgaggctcttacaacgtctcaaccacgggatcacgttatttccactaagtgattggacaaaagtcagattatttagtggaaagtaacgtgattagcaccagtgcgacgccgcgagccccga

SEQ ID NO: 37 - DNA, 170 bp, other sequences
  GTTG PAM containing guide sequence
gtaataaataatatgagttacaggctcatgtcattccgtgcgtgtgctgcgaggctcttacaacgtctcaaccacgggatcacgttatttccactaagtgattggacaaaagtcagattatttagtggaaagtaacgtgattagcacgacgaaaagtttcagtgcgacgc

SEQ ID NO: 38 - DNA, 170 bp, other sequences
  GTTC PAM containing guide sequence
gtaataaataatatgagttacaggctcatgtcattccgtgcgtgtgctgcgaggctcttacaacgtctcaaccacgggatcacgttatttccactaagtgattggacaaaagtcagattatttagtggaaagtaacgtgattagcactcgcttcggaggagccgtggtcc

SEQ ID NO: 39 - protein, 1091 aa, other sequences
  independently identified variant of B-Gen.1 with three amino acid exchanges
MPIRSFKLKLVTHNGDSTYMDKLRRGLWKTHVIINRGIAYYMNTLALMRQEPYGSKSREEVRLDLLSTLREQQRRNNWSEQTGTDDELLSLSRRVYELLVPSAIGEKGDAQMLSRKFLSPLVDPNSEGGRGTAKSGRKPRWKKMMEEGHPDWEKEKEKDAAKKAEDPTASILADLEAVGLLPLFPLFSDEQKEIRWLPKKKRQFVRTWDRDMFQQALERMLSWESWNRRVAEEYQKLQAQRDEVYAKYLEDAGSWLNDLQTFEKQREEELAEVSFEPNSEYLITRRQIRGWKEVYEKWSKTSENASQEQLWRMVADVQTAMAGAFGDPKVYQFLSQPKHHHIWREHPNRLFYYSKYNEVREKLNRAKKQAAFTLPDPVEHPLWTRFDARGGNIHDYEISKVGKQYHVTFSSLILPEAQSWVEIENVTVGIGNSLQLKRQIRLDGYADKKQKVKYYDYSSRFELTGVLGGAKIQFDRKHLKKAAHRLAEGETGPIFLNVVVDVEPFLEVKNGRLRTPLGQVLQVNTRDWPKVVDYKAKELSVLMENTQIGNENGVSTIEAGMRIMSIDLGQRTAAAVSIFEVISKKPDEKETKLFYPIADTDLYAVHRRSLLLRLPGEEISSKKMIEKRKERARIRSLVRYQIRLLSEVLRLHTQGTAEQRRFKLDELLVSIQRKLELDQSEWISELEKLFDYIDESAEKWKEALVVAHRTLEPIVVEAVRNWKKSLSKENKDRRRIAGISIWSIEELEETRKLLIAWSKHSREPGIPKRLEKEETFAPEHLQHIQNVKDDRLKQMANLFVMTALGYKYDEGNKRWVEAYPACQVILFEDLSRYRFALDRPRRENNRLMKWAHRSIPRLTYMQAELFGIQVGDVYSAYTSRFHAKTGAPGIRCHALTEADLQSNSYVVNQLIKDKFIQDNQTEILKAGQIVPWQGGELFVTFADRSGASLAVIHADINAAQNLQKRFWQHNSEVFRVPCKVVKGGLVPVYEKMRKLFGKGLFVNIDDPESKEVYRWEHSTKMKSKTTPVDLESEDIEHEELSDEWEDMQEGYKTLLRDPSGFFWSSDSWIPQKDFWIRVKSRIGKSLREQIR

SEQ ID NO: 40 - RNA, 97 nt, other sequences
  single guide scaffold with N(23) place holder for a target specific sequence B-GEn.1-sgRNA_v4
guuuagcuauaggcuaauaagauaguugugucaagugcuucggagaccuaacacgucauccagucacaacggcuaucuaaaaauagaugguuagcac

SEQ ID NO: 41 - RNA, 87 nt, other sequences
  single guide scaffold with N(23) place holder for a target specific sequence B-GEn.1-sgRNA_v4.2
uuagcuauaggcuaauaagauaguugugucaagugcuucggagaccuaacacgucauccagucacaacggcuaaaaaugguuagcac

SEQ ID NO: 42 - RNA, 87 nt, other sequences
  single guide scaffold with N(23) place holder for a target specific sequence B-GEn.1-sgRNA_v4.3
uuagcuauaggcuaauaagauaguugugucaagugcuucggagaccuaacacgucauccagucacaacggcuaaaaauagccagcac

SEQ ID NO: 43 - RNA, 86 nt, other sequences
  single guide scaffold with N(23) place holder for a target specific sequence B-GEn.1-sgRNA_v4.4
uuagcuauaggcuaauaagauaguugugucaagugcuucggagaccuaacacgucuccagucacaacggcuaaaaauagccagcac

SEQ ID NO: 44 - RNA, 86 nt, other sequences
  single guide scaffold with N(23) place holder for a target specific sequence B-GEn.1-sgRNA_v4.5
uuagcuauaggcuaauaagauaguugugacaagugcuucggagaccuaacacgucuccagucacaacggcuaaaaauagccagcac